European Patent Application EP 4 434 549 A1, published September 25, 2024. Title: 抗体-药物偶联物及其用途. Applicant: 石药集团巨石生物制药有限公司. Application CN. The sequence listing filed with the application follows.

SEQUENCE LISTING (40 sequences)

SEQ ID NO: 1 - protein, 10 aa, synthetic construct
GFNIKDTYIH

SEQ ID NO: 2 - protein, 13 aa, synthetic construct
RIYPTNGYTRYAD

SEQ ID NO: 3 - protein, 11 aa, synthetic construct
WGGDGFYAMDY

SEQ ID NO: 4 - protein, 11 aa, synthetic construct
RASQDVNTAVA

SEQ ID NO: 5 - protein, 7 aa, synthetic construct
SASFLYS

SEQ ID NO: 6 - protein, 9 aa, synthetic construct
QQHYTTPPT

SEQ ID NO: 7 - protein, 120 aa, synthetic construct [sequence omitted]

SEQ ID NO: 8 - protein, 107 aa, synthetic construct [sequence omitted]

SEQ ID NO: 9 - protein, 450 aa, synthetic construct
EVQLVESGGGLVQPGGSLRLSCAASGFNIKDTYIHWVRQAPGKGLEWVARIYPTNGYTRYADSVKGRFTISADTSKNTAYLQMNSLRAEDTAVYYCSRWGGDGFYAMDYWGQGTLVTVSSASTKGPSVFPLAPSSKSTSGGTAALGCLVKDYFPEPVTVSWNSGALTSGVHTFPAVLQSSGLYSLSSVVTVPSSSLGTQTYICNVNHKPSNTKVDKKVEPKSCDKTHTCPPCPAPELLGGPSVFLFPPKPKDTLMISRTPEVTCVVVDVSHEDPEVKFNWYVDGVEVHNAKTKPREEQYNSTYRVVSVLTVLHQDWLNGKEYKCKVSNKALPAPIEKTISKAKGQPREPQVYTLPPSREEMTKNQVSLTCLVKGFYPSDIAVEWESNGQPENNYKTTPPVLDSDGSFFLYSKLTVDKSRWQQGNVFSCSVMHEALHNHYTQKSLSLSPGK

SEQ ID NO: 10 - protein, 214 aa, synthetic construct
DIQMTQSPSSLSASVGDRVTITCRASQDVNTAVAWYQQKPGKAPKLLIYSASFLYSGVPSRFSGSRSGTDFTLTISSLQPEDFATYYCQQHYTTPPTFGQGTKVEIKRTVAAPSVFIFPPSDEQLKSGTASVVCLLNNFYPREAKVQWKVDNALQSGNSQESVTEQDSKDSTYSLSSTLTLSKADYEKHKVYACEVTHQGLSSPVTKSFNRGEC

SEQ ID NO: 11 - protein, 10 aa, synthetic construct
GGSFSGYYWS

SEQ ID NO: 12 - protein, 16 aa, synthetic construct
EINHSGSTNYNPSLKS

SEQ ID NO: 13 - protein, 9 aa, synthetic construct
DKWTWYFDL

SEQ ID NO: 14 - protein, 17 aa, synthetic construct
RSSQSVLYSSSNRNYLA

SEQ ID NO: 15 - protein, 7 aa, synthetic construct
WASTRES

SEQ ID NO: 16 - protein, 9 aa, synthetic construct
QQYYSTPRT

SEQ ID NO: 17 - protein, 117 aa, synthetic construct [sequence omitted]

SEQ ID NO: 18 - protein, 113 aa, synthetic construct [sequence omitted]

SEQ ID NO: 19 - protein, 447 aa, synthetic construct
QVQLQQWGAGLLKPSETLSLTCAVYGGSFSGYYWSWIRQPPGKGLEWIGEINHSGSTNYNPSLKSRVTISVETSKNQFSLKLSSVTAADTAVYYCARDKWTWYFDLWGRGTLVTVSSASTKGPSVFPLAPSSKSTSGGTAALGCLVKDYFPEPVTVSWNSGALTSGVHTFPAVLQSSGLYSLSSVVTVPSSSLGTQTYICNVNHKPSNTKVDKRVEPKSCDKTHTCPPCPAPELLGGPSVFLFPPKPKDTLMISRTPEVTCVVVDVSHEDPEVKFNWYVDGVEVHNAKTKPREEQYNSTYRVVSVLTVLHQDWLNGKEYKCKVSNKALPAPIEKTISKAKGQPREPQVYTLPPSREEMTKNQVSLTCLVKGFYPSDIAVEWESNGQPENNYKTTPPVLDSDGSFFLYSKLTVDKSRWQQGNVFSCSVMHEALHNHYTQKSLSLSPGK

SEQ ID NO: 20 - protein, 220 aa, synthetic construct
DIEMTQSPDSLAVSLGERATINCRSSQSVLYSSSNRNYLAWYQQNPGQPPKLLIYWASTRESGVPDRFSGSGSGTDFTLTISSLQAEDVAVYYCQQYYSTPRTFGQGTKVEIKRTVAAPSVFIFPPSDEQLKSGTASVVCLLNNFYPREAKVQWKVDNALQSGNSQESVTEQDSKDSTYSLSSTLTLSKADYEKHKVYACEVTHQGLSSPVTKSFNRGEC

SEQ ID NO: 21 - protein, 5 aa, synthetic construct
NYDVH

SEQ ID NO: 22 - protein, 16 aa, synthetic construct
VIWSGGNTDYNTPFTS

SEQ ID NO: 23 - protein, 11 aa, synthetic construct
ALDYYDYEFAY

SEQ ID NO: 24 - protein, 11 aa, synthetic construct
RASQSIGTNIH

SEQ ID NO: 25 - protein, 7 aa, synthetic construct
YASESIS

SEQ ID NO: 26 - protein, 9 aa, synthetic construct
QQNNEWPTS

SEQ ID NO: 27 - protein, 119 aa, synthetic construct
QVQLQESGPGLVKPSETLSLTCTVSGFSLSNYDVHWVRQAPGKGLEWLGVIWSGGNTDYNTPFTSRLTISVDTSKNQFSLKLSSVTAADTAVYYCARALDYYDYEFAYWGQGTLVTVSS

SEQ ID NO: 28 - protein, 107 aa, synthetic construct
EIVLTQSPDFQSVTPKEKVTITCRASQSIGTNIHWYQQKPDQSPKLLIKYASESISGIPSRFSGSGSGTDFTLTINSLEAEDAATYYCQQNNEWPTSFGQGTKLEIK

SEQ ID NO: 29 - protein, 449 aa, synthetic construct
QVQLQESGPGLVKPSETLSLTCTVSGFSLSNYDVHWVRQAPGKGLEWLGVIWSGGNTDYNTPFTSRLTISVDTSKNQFSLKLSSVTAADTAVYYCARALDYYDYEFAYWGQGTLVTVSSASTKGPSVFPLAPSSKSTSGGTAALGCLVKDYFPEPVTVSWNSGALTSGVHTFPAVLQSSGLYSLSSVVTVPSSSLGTQTYICNVNHKPSNTKVDKRVEPKSCDKTHTCPPCPAPELLGGPSVFLFPPKPKDTLMISRTPEVTCVVVDVSHEDPEVKFNWYVDGVEVHNAKTKPREEQYNSTYRVVSVLTVLHQDWLNGKEYKCKVSNKALPAPIEKTISKAKGQPREPQVYTLPPSREEMTKNQVSLTCLVKGFYPSDIAVEWESNGQPENNYKTTPPVLDSDGSFFLYSKLTVDKSRWQQGNVFSCSVMHEALHNHYTQKSLSLSPGK

SEQ ID NO: 30 - protein, 214 aa, synthetic construct
EIVLTQSPDFQSVTPKEKVTITCRASQSIGTNIHWYQQKPDQSPKLLIKYASESISGIPSRFSGSGSGTDFTLTINSLEAEDAATYYCQQNNEWPTSFGQGTKLEIKRTVAAPSVFIFPPSDEQLKSGTASVVCLLNNFYPREAKVQWKVDNALQSGNSQESVTEQDSKDSTYSLSSTLTLSKADYEKHKVYACEVTHQGLSSPVTKSFNRGEC

SEQ ID NO: 31 - protein, 5 aa, synthetic construct
DYDVH

SEQ ID NO: 32 - protein, 11 aa, synthetic construct
ALDDYDYEFAY

SEQ ID NO: 33 - protein, 119 aa, synthetic construct
QVQLQESGPGLVKPSETLSLTCTVSGFSLSDYDVHWVRQAPGKGLEWLGVIWSGGNTDYNTPFTSRLTISVDTSKNQFSLKLSSVTAADTAVYYCARALDDYDYEFAYWGQGTLVTVSS

SEQ ID NO: 34 - protein, 449 aa, synthetic construct
QVQLQESGPGLVKPSETLSLTCTVSGFSLSDYDVHWVRQAPGKGLEWLGVIWSGGNTDYNTPFTSRLTISVDTSKNQFSLKLSSVTAADTAVYYCARALDDYDYEFAYWGQGTLVTVSSASTKGPSVFPLAPSSKSTSGGTAALGCLVKDYFPEPVTVSWNSGALTSGVHTFPAVLQSSGLYSLSSVVTVPSSSLGTQTYICNVNHKPSNTKVDKRVEPKSCDKTHTCPPCPAPELLGGPSVFLFPPKPKDTLMISRTPEVTCVVVDVSHEDPEVKFNWYVDGVEVHNAKTKPREEQYNSTYRVVSVLTVLHQDWLNGKEYKCKVSNKALPAPIEKTISKAKGQPREPQVYTLPPSREEMTKNQVSLTCLVKGFYPSDIAVEWESNGQPENNYKTTPPVLDSDGSFFLYSKLTVDKSRWQQGNVFSCSVMHEALHNHYTQKSLSLSPGK

SEQ ID NO: 35 - protein, 5 aa, synthetic construct
EYDVH

SEQ ID NO: 36 - protein, 119 aa, synthetic construct
QVQLQESGPGLVKPSETLSLTCTVSGFSLSEYDVHWVRQAPGKGLEWLGVIWSGGNTDYNTPFTSRLTISVDTSKNQFSLKLSSVTAADTAVYYCARALDDYDYEFAYWGQGTLVTVSS

SEQ ID NO: 37 - protein, 449 aa, synthetic construct
QVQLQESGPGLVKPSETLSLTCTVSGFSLSEYDVHWVRQAPGKGLEWLGVIWSGGNTDYNTPFTSRLTISVDTSKNQFSLKLSSVTAADTAVYYCARALDDYDYEFAYWGQGTLVTVSSASTKGPSVFPLAPSSKSTSGGTAALGCLVKDYFPEPVTVSWNSGALTSGVHTFPAVLQSSGLYSLSSVVTVPSSSLGTQTYICNVNHKPSNTKVDKRVEPKSCDKTHTCPPCPAPELLGGPSVFLFPPKPKDTLMISRTPEVTCVVVDVSHEDPEVKFNWYVDGVEVHNAKTKPREEQYNSTYRVVSVLTVLHQDWLNGKEYKCKVSNKALPAPIEKTISKAKGQPREPQVYTLPPSREEMTKNQVSLTCLVKGFYPSDIAVEWESNGQPENNYKTTPPVLDSDGSFFLYSKLTVDKSRWQQGNVFSCSVMHEALHNHYTQKSLSLSPGK

SEQ ID NO: 38 - protein, 5 aa, synthetic construct
HYDVH

SEQ ID NO: 39 - protein, 119 aa, synthetic construct
QVQLQESGPGLVKPSETLSLTCTVSGFSLSHYDVHWVRQAPGKGLEWLGVIWSGGNTDYNTPFTSRLTISVDTSKNQFSLKLSSVTAADTAVYYCARALDDYDYEFAYWGQGTLVTVSS

SEQ ID NO: 40 - protein, 449 aa, synthetic construct
QVQLQESGPGLVKPSETLSLTCTVSGFSLSHYDVHWVRQAPGKGLEWLGVIWSGGNTDYNTPFTSRLTISVDTSKNQFSLKLSSVTAADTAVYYCARALDDYDYEFAYWGQGTLVTVSSASTKGPSVFPLAPSSKSTSGGTAALGCLVKDYFPEPVTVSWNSGALTSGVHTFPAVLQSSGLYSLSSVVTVPSSSLGTQTYICNVNHKPSNTKVDKRVEPKSCDKTHTCPPCPAPELLGGPSVFLFPPKPKDTLMISRTPEVTCVVVDVSHEDPEVKFNWYVDGVEVHNAKTKPREEQYNSTYRVVSVLTVLHQDWLNGKEYKCKVSNKALPAPIEKTISKAKGQPREPQVYTLPPSREEMTKNQVSLTCLVKGFYPSDIAVEWESNGQPENNYKTTPPVLDSDGSFFLYSKLTVDKSRWQQGNVFSCSVMHEALHNHYTQKSLSLSPGK